European Patent Application EP 4 458 984 A9, published June 4, 2025. Title: 对靶标核酸进行检测的方法. Applicant: 迈克生物股份有限公司. Application CN. The sequence listing filed with the application follows.

SEQUENCE LISTING (39 sequences)

SEQ ID NO: 1 - DNA, 50 bp, synthetic construct
  source 1..50: mol_type = other DNA
tttttctgtcagctgaactggtctcacaaacgcacccagcagtttggccc

SEQ ID NO: 2 - DNA, 32 bp, synthetic construct
  source 1..32: mol_type = other DNA
ccgtgtgcactttcgacctggcagccaggaac

SEQ ID NO: 3 - DNA, 59 bp, synthetic construct
  source 1..59: mol_type = other DNA
gtgcacacggtactgtcagctgaactggtctcactgcagcgctgtccgagctcgacgtg

SEQ ID NO: 4 - DNA, 33 bp, synthetic construct
  source 1..33: mol_type = other DNA
gctcgacgtgaaacgcacccagcagtttggccc

SEQ ID NO: 5 - DNA, 59 bp, synthetic construct
  source 1..59: mol_type = other DNA
ggcttcgagcacttgcactgatccgatcgacgtgcgaccatgacggagagcaggacgag

SEQ ID NO: 6 - DNA, 37 bp, synthetic construct
  source 1..37: mol_type = other DNA
tgctcgaagccaaaagcaaattggacttcccgtaacg

SEQ ID NO: 7 - DNA, 55 bp, synthetic construct
  source 1..55: mol_type = other DNA
ttttttgcactgatccgatcgacgtgctttccttctagagaatgcgtgggaatct

SEQ ID NO: 8 - DNA, 33 bp, synthetic construct
  source 1..33: mol_type = other DNA
tgctcgaagccaaaattggcgaggcacgtatga

SEQ ID NO: 9 - DNA, 37 bp, synthetic construct
  source 1..37: mol_type = other DNA
gcaggacgagtttcaccgtcgagccagaaactgtcta

SEQ ID NO: 10 - DNA, 59 bp, synthetic construct
  source 1..59: mol_type = other DNA
cctcacgctcatgccatatatcaccgtacgtcatcatgccgaacccgatctgctcacca

SEQ ID NO: 11 - DNA, 42 bp, synthetic construct
  source 1..42: mol_type = other DNA
ggcatgagcgtgaggttttagtagtttggctgcctgaaagga

SEQ ID NO: 12 - DNA, 56 bp, synthetic construct
  source 1..56: mol_type = other DNA
ttttttatatcaccgtacgtcatcatgccgaaagtcacccaaattacctagaccgt

SEQ ID NO: 13 - DNA, 37 bp, synthetic construct
  source 1..37: mol_type = other DNA
ggcatgagcgtgaggtttattggcgaggcacgtatga

SEQ ID NO: 14 - DNA, 38 bp, synthetic construct
  source 1..38: mol_type = other DNA
catgccgaaccaaacaccgtcgagccagaaactgtcta

SEQ ID NO: 15 - DNA, 39 bp, synthetic construct
  source 1..39: mol_type = other DNA
ggcatgagcgtgaggtttaaactgacactgggctctgca

SEQ ID NO: 16 - DNA, 33 bp, synthetic construct
  source 1..33: mol_type = other DNA
gctcaccaaaagtcatttgccgtgccatacact

SEQ ID NO: 17 - DNA, 33 bp, synthetic construct
  source 1..33: mol_type = other DNA
gcaggacgagaaacgcacccagcagtttggccc

SEQ ID NO: 18 - DNA, 32 bp, synthetic construct
  source 1..32: mol_type = other DNA
gctcgaagcctttcgacctggcagccaggaac

SEQ ID NO: 19 - DNA, 59 bp, synthetic construct
  source 1..59: mol_type = other DNA
agacgcacggtgacatgtgtttgactcagttctgctgctgcccaccgtctggagtgcgt

SEQ ID NO: 20 - DNA, 36 bp, synthetic construct
  source 1..36: mol_type = other DNA
caccgtgcgtcttttaaactgacactgggctctgca

SEQ ID NO: 21 - DNA, 52 bp, synthetic construct
  source 1..52: mol_type = other DNA
tttttcatgtgtttgactcagttctgcaaagtcatttgccgtgccatacact

SEQ ID NO: 22 - DNA, 39 bp, synthetic construct
  source 1..39: mol_type = other DNA
caccgtgcgtctttttagtagtttggctgcctgaaagga

SEQ ID NO: 23 - DNA, 37 bp, synthetic construct
  source 1..37: mol_type = other DNA
ctggagtgcgtaaagtcacccaaattacctagaccgt

SEQ ID NO: 24 - DNA, 36 bp, synthetic construct
  source 1..36: mol_type = other DNA
ccgtgtgcactttagcaaattggacttcccgtaacg

SEQ ID NO: 25 - DNA, 59 bp, synthetic construct
  source 1..59: mol_type = other DNA
ccctgggagctcatggaatcgctggtcctgtcgacgctgcgcacactgggacggcaccg

SEQ ID NO: 26 - DNA, 51 bp, synthetic construct
  source 1..51: mol_type = other DNA
tttttatggaatcgctggtcctgtcgaaaaagtctgaacgacctacactcc

SEQ ID NO: 27 - DNA, 29 bp, synthetic construct
  source 1..29: mol_type = other DNA
gctcccagggtttcccagcagctgacaca

SEQ ID NO: 28 - DNA, 32 bp, synthetic construct
  source 1..32: mol_type = other DNA
cggcaccgaaaagtctgaacgacctacactcc

SEQ ID NO: 29 - DNA, 54 bp, synthetic construct
  source 1..54: mol_type = other DNA
tttttatggaatcgctggtcctgtcgaaaatattgcagatgtgacaccttagta

SEQ ID NO: 30 - DNA, 42 bp, synthetic construct
  source 1..42: mol_type = other DNA
gctcccagggtttaacctggactaagaagaggaacgacagat

SEQ ID NO: 31 - DNA, 32 bp, synthetic construct
  source 1..32: mol_type = other DNA
gctcccagggtttgactagcaacctccatggc

SEQ ID NO: 32 - DNA, 31 bp, synthetic construct
  source 1..31: mol_type = other DNA
cggcaccgaaaataatcaggcacgagaacag

SEQ ID NO: 33 - DNA, 60 bp, synthetic construct
  source 1..60: mol_type = other DNA
gtcacagctgtcatgaagccgacactgtccgtggagcgacgtggacctctggacgtccgg

SEQ ID NO: 34 - DNA, 47 bp, synthetic construct
  source 1..47: mol_type = other DNA
tttttatgaagccgacactgtccgaaaagactagcaacctccatggc

SEQ ID NO: 35 - DNA, 33 bp, synthetic construct
  source 1..33: mol_type = other DNA
cagctgtgactttataatcaggcacgagaacag

SEQ ID NO: 36 - DNA, 35 bp, synthetic construct
  source 1..35: mol_type = other DNA
gagcgacgtggaaaaatgagaacttgccataggtt

SEQ ID NO: 37 - DNA, 33 bp, synthetic construct
  source 1..33: mol_type = other DNA
cagctgtgactttctaagcagactcacagaact

SEQ ID NO: 38 - DNA, 29 bp, synthetic construct
  source 1..29: mol_type = other DNA
cgtccggtttgcaattcagcatcacagac

SEQ ID NO: 39 - DNA, 35 bp, synthetic construct
  source 1..35: mol_type = other DNA
cagctgtgacaaaaagcaaccaacaacattcattg